European Patent Application EP 4 253 416 A1, published October 4, 2023. Title: ANTI-SIRPa ANTIBODY OR ANTIGEN-BINDING FRAGMENT THEREOF, AND USE THEREOF. Applicant: QURE BIOTECHNOLOGY (SHANGHAI) CO., LTD. Application PCT/CN2021/113416. The sequence listing filed with the application follows.

SEQUENCE LISTING (61 sequences)

SEQ ID NO: 1 - protein, 133 aa, Artificial Sequence
  QP009(SIRPa)
EEELQVIQPDKSVLVAAGETATLRCTATSLIPVGPIQWFRGAGPGRELIYNQKEGHFPRVTTVSDLTKRNNMDFSIRIGNITPADAGTYYCVKFRKGSPDDVEFKSGAGTELSVRAKPSDYKDDDDKHHHHHH

SEQ ID NO: 2 - protein, 119 aa, Artificial Sequence
  71C10 heavy chain variable region
QVQLQQPGTELVRPGASVKLSCKASGYTFTNYWINWVKQRPGQGLEWIAMIDPSDSETHYNQIFKDKATLTVDKSSNTAYMQLSSLTSGDSAVYYCAMDYGSLYAMDYWGRGTSVTVSS

SEQ ID NO: 3 - protein, 5 aa, Artificial Sequence
  71C10 VHCDR1
NYWIN

SEQ ID NO: 4 - protein, 17 aa, Artificial Sequence
  71C10 VHCDR2
MIDPSDSETHYNQIFKD

SEQ ID NO: 5 - protein, 10 aa, Artificial Sequence
  71C10 VHCDR3
DYGSLYAMDY

SEQ ID NO: 6 - protein, 110 aa, Artificial Sequence
  71C10 light chain variable region
DIVLTQSPASLAVSLGQRATISCRASKSVSSSGYNYIFWYQQKPGQPPKLLIYLASNLDSGVPARFSGSGSGTDFTLNIHPVEEEDAATYYCQHSRELPTFGGGTKLEIK

SEQ ID NO: 7 - protein, 15 aa, Artificial Sequence
  71C10 VLCDR1
RASKSVSSSGYNYIF

SEQ ID NO: 8 - protein, 7 aa, Artificial Sequence
  71C10 VLCDR2
LASNLDS

SEQ ID NO: 9 - protein, 8 aa, Artificial Sequence
  71C10 VLCDR3
QHSRELPT

SEQ ID NO: 10 - protein, 237 aa, Artificial Sequence
  QD026 light chain
MDMRVPAQLLGLLLLWFPGSRCQIVLTQSPAIMSASPGEKVTLTCSASSSVSSSYLYWYQQKPGSSPKLWIYSTSNLASGVPARFSGSGSGTSYSLTISSMEAEDAASYFCHQWSSYPRTFGAGTKLELKRTVAAPSVFIFPPSDEQLKSGTASVVCLLNNFYPREAKVQWKVDNALQSGNSQESVTEQDSKDSTYSLSSTLTLSKADYEKHKVYACEVTHQGLSSPVTKSFNRGEC

SEQ ID NO: 11 - protein, 462 aa, Artificial Sequence
  QD027 heavy chain
MEFGLSWLFLVAILKGVQCEVQLQQSGAELVKPGASVKLSCTASGFNIKDYYIHWVQQRTEQGLEWIGRIDPEDGETKYAPKFQDKATITADTSSNTAYLHLSSLTSEDTAVYYCARWGAYWGQGTLVTVSSASTKGPSVFPLAPSSKSTSGGTAALGCLVKDYFPEPVTVSWNSGALTSGVHTFPAVLQSSGLYSLSSVVTVPSSSLGTQTYICNVNHKPSNTKVDKKVEPKSCDKTHTCPPCPAPELLGGPSVFLFPPKPKDTLMISRTPEVTCVVVDVSHEDPEVKFNWYVDGVEVHNAKTKPREEQYNSTYRVVSVLTVLHQDWLNGKEYKCKVSNKALPAPIEKTISKAKGQPREPQVYTLPPSRDELTKNQVSLTCLVKGFYPSDIAVEWESNGQPENNYKTTPPVLDSDGSFFLYSKLTVDKSRWQQGNVFSCSVMHEALHNHYTQKSLSLSPGK

SEQ ID NO: 12 - protein, 459 aa, Artificial Sequence
  QD249 heavy chain
MEFGLSWLFLVAILKGVQCEVQLQQSGAELVKPGASVKLSCTASGFNIKDYYIHWVQQRTEQGLEWIGRIDPEDGETKYAPKFQDKATITADTSSNTAYLHLSSLTSEDTAVYYCARWGAYWGQGTLVTVSSASTKGPSVFPLAPCSRSTSESTAALGCLVKDYFPEPVTVSWNSGALTSGVHTFPAVLQSSGLYSLSSVVTVPSSSLGTKTYTCNVDHKPSNTKVDKRVESKYGPPCPPCPAPEFLGGPSVFLFPPKPKDTLMISRTPEVTCVVVDVSQEDPEVQFNWYVDGVEVHNAKTKPREEQFNSTYRVVSVLTVLHQDWLNGKEYKCKVSNKGLPSSIEKTISKAKGQPREPQVYTLPPSQEEMTKNQVSLTCLVKGFYPSDIAVEWESNGQPENNYKTTPPVLDSDGSFFLYSRLTVDKSRWQEGNVFSCSVMHEALHNHYTQKSLSLSLGK

SEQ ID NO: 13 - protein, 217 aa, Artificial Sequence
  QD163 light chain
DIVLTQSPASLAVSLGQRATISCRASKSVSSSGYNYIFWYQQKPGQPPKLLIYLASNLDSGVPARFSGSGSGTDFTLNIHPVEEEDAATYYCQHSRELPTFGGGTKLEIKRTVAAPSVFIFPPSDEQLKSGTASVVCLLNNFYPREAKVQWKVDNALQSGNSQESVTEQDSKDSTYSLSSTLTLSKADYEKHKVYACEVTHQGLSSPVTKSFNRGEC

SEQ ID NO: 14 - protein, 449 aa, Artificial Sequence
  QD164 heavy chain
QVQLQQPGTELVRPGASVKLSCKASGYTFTNYWINWVKQRPGQGLEWIAMIDPSDSETHYNQIFKDKATLTVDKSSNTAYMQLSSLTSGDSAVYYCAMDYGSLYAMDYWGRGTSVTVSSASTKGPSVFPLAPSSKSTSGGTAALGCLVKDYFPEPVTVSWNSGALTSGVHTFPAVLQSSGLYSLSSVVTVPSSSLGTQTYICNVNHKPSNTKVDKKVEPKSCDKTHTCPPCPAPELLGGPSVFLFPPKPKDTLMISRTPEVTCVVVDVSHEDPEVKFNWYVDGVEVHNAKTKPREEQYNSTYRVVSVLTVLHQDWLNGKEYKCKVSNKALPAPIEKTISKAKGQPREPQVYTLPPSRDELTKNQVSLTCLVKGFYPSDIAVEWESNGQPENNYKTTPPVLDSDGSFFLYSKLTVDKSRWQQGNVFSCSVMHEALHNHYTQKSLSLSPGK

SEQ ID NO: 15 - protein, 465 aa, Artificial Sequence
  QD245 heavy chain
MEFGLSWLFLVAILKGVQCQVQLQQPGTELVRPGASVKLSCKASGYTFTNYWINWVKQRPGQGLEWIAMIDPSDSETHYNQIFKDKATLTVDKSSNTAYMQLSSLTSGDSAVYYCAMDYGSLYAMDYWGRGTSVTVSSASTKGPSVFPLAPCSRSTSESTAALGCLVKDYFPEPVTVSWNSGALTSGVHTFPAVLQSSGLYSLSSVVTVPSSSLGTKTYTCNVDHKPSNTKVDKRVESKYGPPCPPCPAPEFLGGPSVFLFPPKPKDTLMISRTPEVTCVVVDVSQEDPEVQFNWYVDGVEVHNAKTKPREEQFNSTYRVVSVLTVLHQDWLNGKEYKCKVSNKGLPSSIEKTISKAKGQPREPQVYTLPPSQEEMTKNQVSLTCLVKGFYPSDIAVEWESNGQPENNYKTTPPVLDSDGSFFLYSRLTVDKSRWQEGNVFSCSVMHEALHNHYTQKSLSLSLGK

SEQ ID NO: 16 - protein, 110 aa, Artificial Sequence
  QD253 light chain variable region
DIVLTQSPDSLAVSLGERATINCRASKSVSSSGYNYIFWYQQKPGQPPKLLIYLASNLDSGVPDRFSGSGSGTDFTLTISSLQAEDVAVYYCQHSRELPTFGQGTKLEIK

SEQ ID NO: 17 - protein, 119 aa, Artificial Sequence
  QD256 heavy chain variable region
QVQLVQSGAEVKKPGASVKVSCKASGYTFTNYWINWVRQAPGQGLEWIAMIDPSDSETHYNQIFKDRATLTTDTSTSTAYMELRSLRSDDTAVYYCAMDYGSLYAMDYWGRGTLVTVSS

SEQ ID NO: 18 - protein, 110 aa, Artificial Sequence
  QD279 light chain variable region
DIVLTQSPDSLAVSLGERATINCRASQSVRSSGYNWIFWYQQKPGQPPKLLIYLASNRDSGVPDRFSGSGSGTDFTLTISSLQAEDVAVYYCQHSRELPTFGQGTKLEIK

SEQ ID NO: 19 - protein, 110 aa, Artificial Sequence
  QD291 light chain variable region
DIVLTQSPDSLAVSLGERATINCRASKSVGSSGYNWLFWYQQKPGQPPKLLIYLASNRDSGVPDRFSGSGSGTDFTLTISSLQAEDVAVYYCQHSRELPTFGQGTKLEIK

SEQ ID NO: 20 - protein, 110 aa, Artificial Sequence
  QD1581 light chain variable region
DIVLTQSPDSLAVSLGERATINCRASKSVSSSGYNYIFWYQQKPGQPPKLLIYLASNLDPGVPDRFSGSGSGTDFTLTISSLQAEDVAVYYCQHSRELPTFGQGTKLEIK

SEQ ID NO: 21 - protein, 110 aa, Artificial Sequence
  QD1586 light chain variable region
DIVLTQSPDSLAVSLGERATINCRASKSVSSSGYNYIFWYQQKPGQPPKLLIYLASNLDSGVPDRFSGSGSGTDFTLTISSLQAEDVAVYYCQESRELPTFGQGTKLEIK

SEQ ID NO: 22 - protein, 110 aa, Artificial Sequence
  QD1589 light chain variable region
DIVLTQSPDSLAVSLGERATINCRASKSVSSSGYNYIFWYQQKPGQPPKLLIYLASNLDSGVPDRFSGSGSGTDFTLTISSLQAEDVAVYYCQESWELPTFGQGTKLEIK

SEQ ID NO: 23 - protein, 110 aa, Artificial Sequence
  QD1594 light chain variable region
DIVLTQSPDSLAVSLGERATINCRASKSVSSSGYNYIFWYQQKPGQPPKLLIYLASNLDSGVPDRFSGSGSGTDFTLTISSLQAEDVAVYYCQHSRDLPTFGQGTKLEIK

SEQ ID NO: 24 - protein, 110 aa, Artificial Sequence
  QD1770 light chain variable region
DIVLTQSPDSLAVSLGERATINCRASQSVRSSGYNWIFWYQQKPGQPPKLLIYLASNRDSGVPDRFSGSGSGTDFTLTISSLQAEDVAVYYCQESRELPTFGQGTKLEIK

SEQ ID NO: 25 - protein, 110 aa, Artificial Sequence
  QD1771 light chain variable region
DIVLTQSPDSLAVSLGERATINCRASKSVSSSGYNWIFWYQQKPGQPPKLLIYLASNRDSGVPDRFSGSGSGTDFTLTISSLQAEDVAVYYCQESRELPTFGQGTKLEIK

SEQ ID NO: 26 - protein, 449 aa, Artificial Sequence
  QD3270 heavy chain
QVQLVQSGAEVKKPGASVKVSCKASGYTFTNYWINWVRQAPGQGLEWIAMIDPSDSETHYNQIFKDRATLTTDTSTSTAYMELRSLRSDDTAVYYCAMDYGSLYAMDYWGRGTLVTVSSASTKGPSVFPLAPSSKSTSGGTAALGCLVKDYFPEPVTVSWNSGALTSGVHTFPAVLQSSGLYSLSSVVTVPSSSLGTQTYICNVNHKPSNTKVDKKVEPKSCDKTHTCPPCPAPEAAGGPSVFLFPPKPKDTLMISRTPEVTCVVVDVSHEDPEVKFNWYVDGVEVHNAKTKPREEQYNSTYRVVSVLTVLHQDWLNGKEYKCKVSNKALPAPIEKTISAAKGQPREPQVYTLPPSRDELTKNQVSLTCLVKGFYPSDIAVEWESNGQPENNYKTTPPVLDSDGSFFLYSKLTVDKSRWQQGNVFSCSVMHEALHNHYTQKSLSLSPGK

SEQ ID NO: 27 - protein, 449 aa, Artificial Sequence
  QD3225 heavy chain
QVQLVQSGAEVKKPGASVKVSCKASGYTFTNYWINWVRQAPGQGLEWIAMIDPSDSETHYNQIFKDRATLTTDTSTSTAYMELRSLRSDDTAVYYCAMDYGSLYAMDYWGRGTLVTVSSASTKGPSVFPLAPSSKSTSGGTAALGCLVKDYFPEPVTVSWNSGALTSGVHTFPAVLQSSGLYSLSSVVTVPSSSLGTQTYICNVNHKPSNTKVDKKVEPKSCDKTHTCPPCPAPELLGGPSVFLFPPKPKDTLMISRTPEVTCVVVDVSHEDPEVKFNWYVDGVEVHNAKTKPREEQYQSTYRVVSVLTVLHQDWLNGKEYKCKVSNKALPAPIEKTISKAKGQPREPQVYTLPPSRDELTKNQVSLTCLVKGFYPSDIAVEWESNGQPENNYKTTPPVLDSDGSFFLYSKLTVDKSRWQQGNVFSCSVMHEALHNHYTQKSLSLSPGK

SEQ ID NO: 28 - protein, 446 aa, Artificial Sequence
  QD3226 heavy chain
QVQLVQSGAEVKKPGASVKVSCKASGYTFTNYWINWVRQAPGQGLEWIAMIDPSDSETHYNQIFKDRATLTTDTSTSTAYMELRSLRSDDTAVYYCAMDYGSLYAMDYWGRGTLVTVSSASTKGPSVFPLAPCSRSTSESTAALGCLVKDYFPEPVTVSWNSGALTSGVHTFPAVLQSSGLYSLSSVVTVPSSSLGTKTYTCNVDHKPSNTKVDKRVESKYGPPCPPCPAPEFLGGPSVFLFPPKPKDTLMISRTPEVTCVVVDVSQEDPEVQFNWYVDGVEVHNAKTKPREEQFQSTYRVVSVLTVLHQDWLNGKEYKCKVSNKGLPSSIEKTISKAKGQPREPQVYTLPPSQEEMTKNQVSLTCLVKGFYPSDIAVEWESNGQPENNYKTTPPVLDSDGSFFLYSRLTVDKSRWQEGNVFSCSVMHEALHNHYTQKSLSLSLGK

SEQ ID NO: 29 - protein, 445 aa, Artificial Sequence
  QD3255 heavy chain
QVQLVQSGAEVKKPGASVKVSCKASGYTFTNYWINWVRQAPGQGLEWIAMIDPSDSETHYNQIFKDRATLTTDTSTSTAYMELRSLRSDDTAVYYCAMDYGSLYAMDYWGRGTLVTVSSASTKGPSVFPLAPCSRSTSESTAALGCLVKDYFPEPVTVSWNSGALTSGVHTFPAVLQSSGLYSLSSVVTVPSSNFGTQTYTCNVDHKPSNTKVDKTVERKCCVECPPCPAPPVAGPSVFLFPPKPKDTLMISRTPEVTCVVVDVSHEDPEVQFNWYVDGVEVHNAKTKPREEQFNSTFRVVSVLTVVHQDWLNGKEYKCKVSNKGLPAPIEKTISKTKGQPREPQVYTLPPSREEMTKNQVSLTCLVKGFYPSDIAVEWESNGQPENNYKTTPPMLDSDGSFFLYSKLTVDKSRWQQGNVFSCSVMHEALHNHYTQKSLSLSPGK

SEQ ID NO: 30 - protein, 449 aa, Artificial Sequence
  QD3260 heavy chain
QVQLVQSGAEVKKPGASVKVSCKASGYTFTNYWINWVRQAPGQGLEWIAMIDPSDSETHYNQIFKDRATLTTDTSTSTAYMELRSLRSDDTAVYYCAMDYGSLYAMDYWGRGTLVTVSSASTKGPSVFPLAPSSKSTSGGTAALGCLVKDYFPEPVTVSWNSGALTSGVHTFPAVLQSSGLYSLSSVVTVPSSSLGTQTYICNVNHKPSNTKVDKKVEPKSCDKTHTCPPCPAPEAAGGPSVFLFPPKPKDTLMISRTPEVTCVVVDVSHEDPEVKFNWYVDGVEVHNAKTKPREEQYNSTYRVVSVLTVLHQDWLNGKEYKCKVSNKALPAPIEKTISKAKGQPREPQVYTLPPSRDELTKNQVSLTCLVKGFYPSDIAVEWESNGQPENNYKTTPPVLDSDGSFFLYSKLTVDKSRWQQGNVFSCSVMHEALHNHYTQKSLSLSPGK

SEQ ID NO: 31 - protein, 449 aa, Artificial Sequence
  QD3265 heavy chain
QVQLVQSGAEVKKPGASVKVSCKASGYTFTNYWINWVRQAPGQGLEWIAMIDPSDSETHYNQIFKDRATLTTDTSTSTAYMELRSLRSDDTAVYYCAMDYGSLYAMDYWGRGTLVTVSSASTKGPSVFPLAPSSKSTSGGTAALGCLVKDYFPEPVTVSWNSGALTSGVHTFPAVLQSSGLYSLSSVVTVPSSSLGTQTYICNVNHKPSNTKVDKKVEPKSCDKTHTCPPCPAPEAAGGPSVFLFPPKPKDTLMISRTPEVTCVVVDVSHEDPEVKFNWYVDGVEVHNAKTKPREEQYNSTYRVVSVLTVLHQDWLNGKEYKCKVSNKALGAPIEKTISKAKGQPREPQVYTLPPSRDELTKNQVSLTCLVKGFYPSDIAVEWESNGQPENNYKTTPPVLDSDGSFFLYSKLTVDKSRWQQGNVFSCSVMHEALHNHYTQKSLSLSPGK

SEQ ID NO: 32 - protein, 443 aa, Artificial Sequence
  QD3268 heavy chain
EVQLQQSGAELVKPGASVKLSCTASGFNIKDYYIHWVQQRTEQGLEWIGRIDPEDGETKYAPKFQDKATITADTSSNTAYLHLSSLTSEDTAVYYCARWGAYWGQGTLVTVSSASTKGPSVFPLAPSSKSTSGGTAALGCLVKDYFPEPVTVSWNSGALTSGVHTFPAVLQSSGLYSLSSVVTVPSSSLGTQTYICNVNHKPSNTKVDKKVEPKSCDKTHTCPPCPAPEAAGGPSVFLFPPKPKDTLMISRTPEVTCVVVDVSHEDPEVKFNWYVDGVEVHNAKTKPREEQYNSTYRVVSVLTVLHQDWLNGKEYKCKVSNKALPAPIEKTISAAKGQPREPQVYTLPPSRDELTKNQVSLTCLVKGFYPSDIAVEWESNGQPENNYKTTPPVLDSDGSFFLYSKLTVDKSRWQQGNVFSCSVMHEALHNHYTQKSLSLSPGK

SEQ ID NO: 33 - protein, 449 aa, Artificial Sequence
  QD3271 heavy chain
QVQLQQSGPELVKPGASVRISCKASGFTFTNYYIHWVKQRPGQGLEWIGWIYPGNVNTKYNEKFKAKATLTADKSSTTAYMQLSSLASEDSAVYFCARPTIIATDFDVWGAGTTVTVSSASTKGPSVFPLAPSSKSTSGGTAALGCLVKDYFPEPVTVSWNSGALTSGVHTFPAVLQSSGLYSLSSVVTVPSSSLGTQTYICNVNHKPSNTKVDKKVEPKSCDKTHTCPPCPAPEAAGGPSVFLFPPKPKDTLMISRTPEVTCVVVDVSHEDPEVKFNWYVDGVEVHNAKTKPREEQYNSTYRVVSVLTVLHQDWLNGKEYKCKVSNKALPAPIEKTISAAKGQPREPQVYTLPPSRDELTKNQVSLTCLVKGFYPSDIAVEWESNGQPENNYKTTPPVLDSDGSFFLYSKLTVDKSRWQQGNVFSCSVMHEALHNHYTQKSLSLSPGK

SEQ ID NO: 34 - protein, 449 aa, Artificial Sequence
  QD3222 heavy chain
QVQLQQPGTELVRPGASVKLSCKASGYTFTNYWINWVKQRPGQGLEWIAMIDPSDSETHYNQIFKDKATLTVDKSSNTAYMQLSSLTSGDSAVYYCAMDYGSLYAMDYWGRGTSVTVSSASTKGPSVFPLAPSSKSTSGGTAALGCLVKDYFPEPVTVSWNSGALTSGVHTFPAVLQSSGLYSLSSVVTVPSSSLGTQTYICNVNHKPSNTKVDKKVEPKSCDKTHTCPPCPAPELLGGPSVFLFPPKPKDTLMISRTPEVTCVVVDVSHEDPEVKFNWYVDGVEVHNAKTKPREEQYQSTYRVVSVLTVLHQDWLNGKEYKCKVSNKALPAPIEKTISKAKGQPREPQVYTLPPSRDELTKNQVSLTCLVKGFYPSDIAVEWESNGQPENNYKTTPPVLDSDGSFFLYSKLTVDKSRWQQGNVFSCSVMHEALHNHYTQKSLSLSPGK

SEQ ID NO: 35 - protein, 440 aa, Artificial Sequence
  QD3221 heavy chain
EVQLQQSGAELVKPGASVKLSCTASGFNIKDYYIHWVQQRTEQGLEWIGRIDPEDGETKYAPKFQDKATITADTSSNTAYLHLSSLTSEDTAVYYCARWGAYWGQGTLVTVSSASTKGPSVFPLAPCSRSTSESTAALGCLVKDYFPEPVTVSWNSGALTSGVHTFPAVLQSSGLYSLSSVVTVPSSSLGTKTYTCNVDHKPSNTKVDKRVESKYGPPCPPCPAPEFLGGPSVFLFPPKPKDTLMISRTPEVTCVVVDVSQEDPEVQFNWYVDGVEVHNAKTKPREEQFQSTYRVVSVLTVLHQDWLNGKEYKCKVSNKGLPSSIEKTISKAKGQPREPQVYTLPPSQEEMTKNQVSLTCLVKGFYPSDIAVEWESNGQPENNYKTTPPVLDSDGSFFLYSRLTVDKSRWQEGNVFSCSVMHEALHNHYTQKSLSLSLGK

SEQ ID NO: 36 - protein, 236 aa, Artificial Sequence
  QD3240 light chain
MDMRVPAQLLGLLLLWFPGSRCDIVMTQSHKFMSTSVGDRVNITCKASQGVGTAVGWYQQKPGQSPRLLIYWASTRHTGVPDRFTGSGSGTDFSLAISNVQSEDLADYFCQQYSTYPFTFGGGTNLEIKRTVAAPSVFIFPPSDEQLKSGTASVVCLLNNFYPREAKVQWKVDNALQSGNSQESVTEQDSKDSTYSLSSTLTLSKADYEKHKVYACEVTHQGLSSPVTKSFNRGEC

SEQ ID NO: 37 - protein, 15 aa, Artificial Sequence
  QD279/QD1770 VLCDR1
RASQSVRSSGYNWIF

SEQ ID NO: 38 - protein, 7 aa, Artificial Sequence
  QD279/QD291/QD1770/QD1771 VLCDR2
LASNRDS

SEQ ID NO: 39 - protein, 15 aa, Artificial Sequence
  QD291 VLCDR1
RASKSVGSSGYNWLF

SEQ ID NO: 40 - protein, 7 aa, Artificial Sequence
  QD1581 VLCDR2
LASNLDP

SEQ ID NO: 41 - protein, 8 aa, Artificial Sequence
  QD1586/QD1770/QD1771 VLCDR3
QESRELPT

SEQ ID NO: 42 - protein, 8 aa, Artificial Sequence
  QD1589 VLCDR3
QESWELPT

SEQ ID NO: 43 - protein, 8 aa, Artificial Sequence
  QD1594 VLCDR3
QHSRDLPT

SEQ ID NO: 44 - protein, 15 aa, Artificial Sequence
  QD1771 VLCDR1
RASKSVSSSGYNWIF

SEQ ID NO: 45 - protein, 376 aa, Artificial Sequence
  QP094
MEFGLSWLFLVAILKGVQCEEELQVIQPDKSVLVAAGETATLRCTATSLIPVGPIQWFRGAGPGRELIYNQKEGHFPRVTTVSDLTKRNNMDFSIRIGNITPADAGTYYCVKFRKGSPDDVEFKSGAGTELSVRAKPSAPVVSGPAARATPQHTVSFTCESHGFSPRDITLKWFKNGNELSDFQTNVDPVGESVSYSIHSTAKVVLTREDVHSQVICEVAHVTLQGDPLRGTANLSETIRVPPTLEVTQQPVRAENQVNVTCQVRKFYPQRLQLTWLENGNVSRTETASTVTENKDGTYNWMSWLLVNVSAHRDDVKLTCQVEHDGQPAVSKSHDLKVSAHPKEQGSNTAAENTGSNERGSSDYKDDDDKHHHHHH

SEQ ID NO: 46 - protein, 375 aa, Artificial Sequence
  QP096
MEFGLSWLFLVAILKGVQCEEELQVIQPDKSVSVAAGESAILHCTVTSLIPVGPIQWFRGAGPARELIYNQKEGHFPRVTTVSESTKRENMDFSISISNITPADAGTYYCVKFRKGSPDTEFKSGAGTELSVRAKPSAPVVSGPAARATPQHTVSFTCESHGFSPRDITLKWFKNGNELSDFQTNVDPVGESVSYSIHSTAKVVLTREDVHSQVICEVAHVTLQGDPLRGTANLSETIRVPPTLEVTQQPVRAENQVNVTCQVRKFYPQRLQLTWLENGNVSRTETASTVTENKDGTYNWMSWLLVNVSAHRDDVKLTCQVEHDGQPAVSKSHDLKVSAHPKEQGSNTAAENTGSNERGSSDYKDDDDKHHHHHH

SEQ ID NO: 47 - protein, 375 aa, Artificial Sequence
  QP098
MEFGLSWLFLVAILKGVQCEEELQVIQPEKSVSVAAGDSATLNCTVSSLIPVGPIQWFRGAGPGRELIYNLKEGHFPRVTAVSDPTKRNNMDFSIRISNITPADAGTYYCVKFRKGSPDVELKSGAGTELSVRAKPSAPVVSGPAVRATAEHTVSFTCESHGFSPRDITLKWFKNGNELSDVQTNVDPAGKSVSYSIRSTARVLLTRRDVHSQVICEVAHVTLQGDPLRGTANLSEAIRVPPFLEVTQQSMRADNQVNVTCQVTKFYPQRLQLTWLENGNVSRTEMASALPENKDGTYNWTSWLLVNVSAHRDDVKLTCQVEHDGQPAVNKSFSVKVSAHPKEQGSNTAAENTGTNERGSSDYKDDDDKHHHHHH

SEQ ID NO: 48 - protein, 375 aa, Artificial Sequence
  QP100
MEFGLSWLFLVAILKGVQCEEELQVIQPEKSVSVAAGESATLNCTATSLIPVGPIQWFRGVGPGRELIYHQKEGHFPRVTPVSDPTKRNNMDFSIRISNITPADAGTYYCVKFRKGSPDVELKSGAGTELSVRAKPSAPVVSGPAVRATAEHTVSFTCESHGFSPRDITLKWFKNGNELSDFQTNVDPAGKSVSYSIRSTARVVLTRRDVHSQVICEVAHVTLQGDPLRGTANLSEAIRVPPFLEFTQQSMRADNQVNVTCQVMKFYPQRLQLTWLENGNVSRTEMASALPENKDGTYNWTSWLLVNVSAHRDDVKLTCQVEHDGQPAVNKSFSVKVSAHPKEQGSNTAAENTGTNERGSSDYKDDDDKHHHHHH

SEQ ID NO: 49 - protein, 372 aa, Artificial Sequence
  QP271
MEFGLSWLFLVAILKGVQCEEELQVIQPEKSVSVAAGDSATLNCTVTSLIPVGPIQWFRGAGPGRELIYHQKEGHFPRVTSVSESTKRNNMDFSIHISNITPADAGTYYCVKFRKGSPDVEVKSGAGTELSVRAKPSAPVVSGPAVRATAEHTVSFTCESHGFSPRDITLKWFKNGNELSDFQTNVDPAGKSVSYSIRSTARVVLTRRDVHSQVICEVAHVTLQGDPLRGTANLSEAIRVPPFLEVTQQSMRADNQVNVTCQVTKFYPQRLQLTWLENGNVSRTEMASALPENKDGTYNWTSWLLVNVSAHRDDVKLTCQVEHDGQPAVNKSFSVKVSAHPKEQGSNTAAENTGTNERDYKDDDDKHHHHHH

SEQ ID NO: 50 - protein, 372 aa, Artificial Sequence
  QP273
MEFGLSWLFLVAILKGVQCEEELQVIQPEKSVSVAAGESATLNCTATSLIPVGPIQWFRGVGPGRELIYSQKEGHFPRVTPVSDPTKRNNMDFSIRISNITPADAGTYYCVKFRKGSPDVELKSGAGTELSVRAKPSAPVVSGPAVRATAEHTVSFTCESHGFSPRDITLKWFKNGNELSDFQTNVDPAGKSVSYSIRSTARVVLTRRDVHSQVICEVAHVTLQGDPLRGTANLSEAIRVPPFLEVTQQSMRADNQVNVTCQVTKFYPQRLQLTWLENGNVSRTEMASALPENKDGTYNWTSWLLVNVSAHRDDVKLTCQVEHDGQPAVNKSFSVKVSAHPKEQGSNTAAENTGTNERDYKDDDDKHHHHHH

SEQ ID NO: 51 - protein, 123 aa, Artificial Sequence
  SIRPa V1
GVAGEEELQVIQPDKSVLVAAGETATLRCTATSLIPVGPIQWFRGAGPGRELIYNQKEGHFPRVTTVSDLTKRNNMDFSIRIGNITPADAGTYYCVKFRKGSPDDVEFKSGAGTELSVRAKPS

SEQ ID NO: 52 - protein, 122 aa, Artificial Sequence
  SIRPa V2
GVAGEEELQVIQPDKSVSVAAGESAILHCTVTSLIPVGPIQWFRGAGPARELIYNQKEGHFPRVTTVSESTKRENMDFSISISNITPADAGTYYCVKFRKGSPDTEFKSGAGTELSVRAKPS

SEQ ID NO: 53 - protein, 122 aa, Artificial Sequence
  SIRPa V3
GVAGEEELQVIQPDKSVSVAAGESAILLCTVTSLIPVGPIQWFRGAGPARELIYNQKEGHFPRVTTVSESTKRENMDFSISISNITPADAGTYYCVKFRKGSPDTEFKSGAGTELSVRAKPS

SEQ ID NO: 54 - protein, 123 aa, Artificial Sequence
  SIRPa V4
GVAGEEGLQVIQPDKSVSVAAGESAILHCTATSLIPVGPIQWFRGAGPGRELIYNQKEGHFPRVTTVSDLTKRNNMDFSIRIGNITPADAGTYYCVKFRKGSPDDVEFKSGAGTELSVRAKPS

SEQ ID NO: 55 - protein, 123 aa, Artificial Sequence
  SIRPa V5
GVAGEEELQVIQPDKFVLVAAGETATLRCTATSLIPVGPIQWFRGAGPGRELIYNQKEGHFPRVTTVSDLTKRNNMDFSIRIGNITPADAGTYYCVKFRKGSPDDVEFKSGAGTELSVRAKPS

SEQ ID NO: 56 - protein, 123 aa, Artificial Sequence
  SIRPa V6
GVAGEEELQVIQPDKSVLVAAGETATLRCTATSLIPVGPIQWFRGAGPGRELIYNQKEGHFPRVTTVSDLTKRNNMDFPIRIGNITPADAGTYYCVKFRKGSPDDVEFKSGAGTELSVRAKPS

SEQ ID NO: 57 - protein, 122 aa, Artificial Sequence
  SIRPa V7
GVAGEEELQVIQPDKSVSVAAGESAILHCTVTSLIPVGPIQWFRGAGPARELIYNQKEGHFPRVTTVSESTKRENMDFSISISNITPADAGTYYCVKFRKGSPDTEFKSGAGTELSVRGKPS

SEQ ID NO: 58 - protein, 122 aa, Artificial Sequence
  SIRPa V8
GVAGEEELQVIQPDKSVLVAAGETATLRCTATSLIPVGPIQWFRGAGPARELIYNQKEGHFPRVTTVSESTKRENMDFSISISNITPADAGTYYCVKFRKGSPDTEFKSGAGTELSVRAKPS

SEQ ID NO: 59 - protein, 123 aa, Artificial Sequence
  SIRPa V9
GVAGEEELQVIQPDKSVLVAAGETATLRCTATSLIPVGPIQWFRGAGPGRELIYNQKEGHFPRVTTVSDLTKRNNMDFSIRISNITPADAGTYYCVKFRKGSPDDVEFKSGAGTELSVRAKPS

SEQ ID NO: 60 - protein, 122 aa, Artificial Sequence
  SIRPa V10
RVAGEEELQVIQPDKSVSVAAGESAILHCTVTSLIPVGPIQWFRGAGPARELIYNQKEGHFPRVTTVSESTKRENMDFSISISNITPADAGTYYCVKFRKGSPDTEFKSGAGTELSVRAKPS

SEQ ID NO: 61 - protein, 233 aa, Artificial Sequence
  FC(mouse IgG2a)
EPRGPTIKPCPPCKCPAPNLLGGPSVFIFPPKIKDVLMISLSPIVTCVVVDVSEDDPDVQISWFVNNVEVHTAQTQTHREDYNSTLRVVSALPIQHQDWMSGKEFKCKVNNKDLPAPIERTISKPKGSVRAPQVYVLPPPEEEMTKKQVTLTCMVTDFMPEDIYVEWTNNGKTELNYKNTEPVLDSDGSYFMYSKLRVEKKNWVERNSYSCSVVHEGLHNHHTTKSFSRTPGK